European Patent Application EP 4 129 326 A1, published February 8, 2023. Title: Recombinant Protein for Animal Neutering and Vaccine Composition Comprising the Same. Applicant: BioApplications Inc. The sequence listing filed with the application follows.

SEQUENCE LISTING (13 sequences)

SEQ ID NO: 1 - protein, 10 aa, Artificial Sequence
  Amino acid sequence of GnRH
EHWSYGLRPG

SEQ ID NO: 2 - protein, 78 aa, Artificial Sequence
  Amino acid sequence of 6X GnRH
AGAEHWSYGLRPGAGAEHWSYGLRPGAGAEHWSYGLRPGAGAEHWSYGLRPGAGAEHWSYGLRPGAGAEHWSYGLRPG

SEQ ID NO: 3 - DNA, 234 bp, Artificial Sequence
  DNA sequence of 6X GnRH
gcaggagcagaacattggtcttacggtcttagacctggagctggagctgaacattggagttatggtttaagacctggagctggagctgaacattggtcttatggacttagaccaggtgcaggtgctgagcattggtcatatggattgagaccaggagctggtgctgagcattggtcttatggtctaagacctggagctggagctgaacattggtcttacggactcagacccggt

SEQ ID NO: 4 - protein, 102 aa, Artificial Sequence
  Amino acid sequence of CTB
TPQNITDLCAEYHNTQIHTLNDKIFSYTESLAGKREMAIITFKNGATFQVEVPGSQHIDSQKKAIERMKDTLRIAYLTEAKVEKLCVWNNKTPHAIAAISMA

SEQ ID NO: 5 - DNA, 306 bp, Artificial Sequence
  DNA sequence of CTB
actcctcagaacataaccgatttgtgcgctgaataccataacactcaaatacacacactcaacgataagattttctcttacactgaatcacttgctggaaagagagagatggcaattatcacctttaaaaacggagctactttccaggttgaagtgcctggtagtcaacatatcgattcacagaagaaagcaatagagaggatgaaggatacacttaggattgcttatttgaccgaagcaaaagttgagaaactctgtgtgtggaataacaaaacccctcacgctatcgctgctatctctatggcc

SEQ ID NO: 6 - protein, 229 aa, Artificial Sequence
  Amino acid sequence of pFc2
RAVGRPCPICPACEGPGPSAFIFPPKPKDTLMISRTPQVTCVVVDVSQENPEVQFSWYVDGVEVHTAQTRPKEAQFNSTYRVVSVLPIQHEDWLKGKEFECKVNNKDLPAPITRIISKAKGPSREPQVYTLSPSAEELSRSKVSITCLVTGFYPPDIDVEWKSNGQPEPEGNYRTTPPQQDVDGTYFLYSKLAVDKASWQRGDPFQCAVMHEALHNHYTQKSVSKTQGK

SEQ ID NO: 7 - DNA, 681 bp, Artificial Sequence
  DNA sequence of pFc2
gttggaagaccatgccctatatgtcctgcttgtgaaggtccaggtccctctgcttttatattcccaccaaagccgaaggataccttgatgatttcacgtacaccacaagttacttgtgttgttgtggatgtttcacaagaaaatcctgaggtacaattcagctggtatgttgatggggtagaagtgcacactgcacagactcgaccaaaggaggcccagtttaactcgacttatagagttgtttctgttctcccaatccaacacgaagattggctgaagggcaaggaatttgaatgcaaggttaacaataaagatctaccagcaccaattaccaggattatttctaaggcaaaaggaccctccagagagccccaagtttacacattgtctccttctgctgaggagcttagtagaagtaaagtgagcattacctgcttagtgacgggattctaccctccagacatcgacgtcgaatggaaatctaatggtcaacctgagccagaaggtaactataggactactccaccacaacaggacgtcgatggcacatactttctttattcaaaacttgctgtcgataaggcaagttggcaaagaggagatccatttcagtgtgctgtaatgcatgaggctttgcataatcattatacacagaaatcagtttctaaaacacaagggaaa

SEQ ID NO: 8 - protein, 7 aa, Artificial Sequence
  Amino acid sequence of BiP
IEEATKL

SEQ ID NO: 9 - DNA, 273 bp, Artificial Sequence
  DNA sequence of BiP
atggctcgctcgtttggagctaacagtaccgttgtgttggcgatcatcttcttcggtgagtgattttccgatcttcttctccgatttagatctcctctacattgttgcttaatctcagaaccttttttcgttgttcctggatctgaatgtgtttgtttgcaatttcacgatcttaaaaggttagatctcgattggtattgacgattggaatctttacgatttcaggatgtttatttgcgttgtcctctgcaatagaagaggctacgaagttaa

SEQ ID NO: 10 - protein, 4 aa, Artificial Sequence
  Amino acid sequence of HDEL
HDEL

SEQ ID NO: 11 - DNA, 12 bp, Artificial Sequence
  DNA sequence of HDEL
cacgatgagctc

SEQ ID NO: 12 - protein, 428 aa, Artificial Sequence
  Full amino acid sequence of 1300-BiP:CTB:GnRH:pFc2:HDEL
IEEATKLRILTPQNITDLCAEYHNTQIHTLNDKIFSYTESLAGKREMAIITFKNGATFQVEVPGSQHIDSQKKAIERMKDTLRIAYLTEAKVEKLCVWNNKTPHAIAAISMATSAGAEHWSYGLRPGAGAEHWSYGLRPGAGAEHWSYGLRPGAGAEHWSYGLRPGAGAEHWSYGLRPGAGAEHWSYGLRPGARARAVGRPCPICPACEGPGPSAFIFPPKPKDTLMISRTPQVTCVVVDVSQENPEVQFSWYVDGVEVHTAQTRPKEAQFNSTYRVVSVLPIQHEDWLKGKEFECKVNNKDLPAPITRIISKAKGPSREPQVYTLSPSAEELSRSKVSITCLVTGFYPPDIDVEWKSNGQPEPEGNYRTTPPQQDVDGTYFLYSKLAVDKASWQRGDPFQCAVMHEALHNHYTQKSVSKTQGKHDEL

SEQ ID NO: 13 - DNA, 1565 bp, Artificial Sequence
  Full DNA sequence of 1300-BiP:CTB:GnRH:pFc2:HDEL
tctagaattattacatcaaaacaaaaaatggctcgctcgtttggagctaacagtaccgttgtgttggcgatcatcttcttcggtgagtgattttccgatcttcttctccgatttagatctcctctacattgttgcttaatctcagaaccttttttcgttgttcctggatctgaatgtgtttgtttgcaatttcacgatcttaaaaggttagatctcgattggtattgacgattggaatctttacgatttcaggatgtttatttgcgttgtcctctgcaatagaagaggctacgaagttaaggatcctcactcctcagaacataaccgatttgtgcgctgaataccataacactcaaatacacacactcaacgataagattttctcttacactgaatcacttgctggaaagagagagatggcaattatcacctttaaaaacggagctactttccaggttgaagtgcctggtagtcaacatatcgattcacagaagaaagcaatagagaggatgaaggatacacttaggattgcttatttgaccgaagcaaaagttgagaaactctgtgtgtggaataacaaaacccctcacgctatcgctgctatctctatggccactagtgcaggagcagaacattggtcttacggtcttagacctggagctggagctgaacattggagttatggtttaagacctggagctggagctgaacattggtcttatggacttagaccaggtgcaggtgctgagcattggtcatatggattgagaccaggagctggtgctgagcattggtcttatggtctaagacctggagctggagctgaacattggtcttacggactcagacccggtgcccgggcagttggaagaccatgccctatatgtcctgcttgtgaaggtccaggtccctctgcttttatattcccaccaaagccgaaggataccttgatgatttcacgtacaccacaagttacttgtgttgttgtggatgtttcacaagaaaatcctgaggtacaattcagctggtatgttgatggggtagaagtgcacactgcacagactcgaccaaaggaggcccagtttaactcgacttatagagttgtttctgttctcccaatccaacacgaagattggctgaagggcaaggaatttgaatgcaaggttaacaataaagatctaccagcaccaattaccaggattatttctaaggcaaaaggaccctccagagagccccaagtttacacattgtctccttctgctgaggagcttagtagaagtaaagtgagcattacctgcttagtgacgggattctaccctccagacatcgacgtcgaatggaaatctaatggtcaacctgagccagaaggtaactataggactactccaccacaacaggacgtcgatggcacatactttctttattcaaaacttgctgtcgataaggcaagttggcaaagaggagatccatttcagtgtgctgtaatgcatgaggctttgcataatcattatacacagaaatcagtttctaaaacacaagggaaacacgatgagctctagctcgag